European Patent Application EP 4 296 276 A1, published December 27, 2023. Title: DISC1-binding peptides and the use thereof for the treatment and diagnosis of schizophrenia and other chronic mental disorders. Applicant: Forschungszentrum Juelich GmbH. The sequence listing filed with the application follows.

SEQUENCE LISTING (12 sequences)

SEQ ID NO: 1 - protein, 16 aa, Artificial Sequence
  Peptide
IWAGHIHDWWRRGQGS

SEQ ID NO: 2 - protein, 16 aa, Artificial Sequence
  Peptide
AWQHHELKWKQYQGWR

SEQ ID NO: 3 - protein, 16 aa, Artificial Sequence
  Peptide
GIKSLISNKMHTQWNY

SEQ ID NO: 4 - protein, 16 aa, Artificial Sequence
  Peptide
WNHPMNIRSISWHKDS

SEQ ID NO: 5 - protein, 16 aa, Artificial Sequence
  Peptide
PWYNAPHSHGFWGSGR

SEQ ID NO: 6 - protein, 16 aa, Artificial Sequence
  Peptide
HKLHHLLKWENQHKVE

SEQ ID NO: 7 - protein, 16 aa, Artificial Sequence
  Peptide
FPHPTLKHREFMRHVS

SEQ ID NO: 8 - protein, 16 aa, Artificial Sequence
  Peptide
HISMQTYKWSQWAKHQ

SEQ ID NO: 9 - protein, 16 aa, Artificial Sequence
  Peptide
QDNPWWHEHKHWKSWP

SEQ ID NO: 10 - protein, 16 aa, Artificial Sequence
  Peptide
SNWHPRHFFMSPSSPQ

SEQ ID NO: 11 - protein, 16 aa, Artificial Sequence
  Peptide
KYTAIHEWYKAHNGGA

SEQ ID NO: 12 - protein, 16 aa, Artificial Sequence
  Peptide
TSGVPWWKFQQQVRRT